European Patent Application EP 4 169 941 A1, published April 26, 2023. Title: Method for detecting adenocarcinoma. Applicant: MITSUI CHEMICALS, INC. The sequence listing filed with the application follows.

SEQUENCE LISTING (10 sequences)

SEQ ID NO: 1 - protein, 61 aa, Homo sapiens
EKTGVCPELQADQNCTQECVSDSECADNLKCCSAGCATFCSLPNDKEGSCPQVNINFPQLG

SEQ ID NO: 2 - protein, 56 aa, Homo sapiens
EKTGVCPELQADQNCTQECVSDSECADNLKCCSAGCATFCSLPNDKEGSCPQVNIN

SEQ ID NO: 3 - protein, 94 aa, Homo sapiens
EKTGVCPELQADQNCTQECVSDSECADNLKCCSAGCATFCSLPNDKEGSCPQVNINFPQLGLCRDQCQVDSQCPGQMKCCRNGCGKVSCVTPNF

SEQ ID NO: 4 - protein, 64 aa, Artificial Sequence
  synthetic peptide
TGAEKTGVCPELQADQNCTQECVSDSECADNLKCCSAGCATFCSLPNDKEGSSPQVNINFPQLG

SEQ ID NO: 5 - protein, 59 aa, Artificial Sequence
  synthetic peptide
TGAEKTGVCPELQADQNCTQECVSDSECADNLKCCSAGCATFCSLPNDKEGSSPQVNIN

SEQ ID NO: 6 - protein, 97 aa, Artificial Sequence
  synthetic peptide
TGAEKTGVCPELQADQNCTQECVSDSECADNLKCCSAGCATFCSLPNDKEGSCPQVNINFPQLGLCRDQCQVDSQCPGQMKCCRNGCGKVSCVTPNF

SEQ ID NO: 7 - protein, 8 aa, Artificial Sequence
  sythetic peptide
CGGGPQLG

SEQ ID NO: 8 - protein, 9 aa, Artificial Sequence
  synthetic peptide
CGGGQVNIN

SEQ ID NO: 9 - protein, 8 aa, Artificial Sequence
  synthetic peptide
CGGGTPNF

SEQ ID NO: 10 - protein, 31 aa, Artificial Sequence
  synthetic peptide
RDQCQVDSQCPGQMKCCRNGCGKVSCVTPNF